European Patent Application EP 4 722 234 A1, published April 8, 2026. Title: GENE CONSTRUCT COMPRISING A NUCLEOTIDES ENCODING DECOY PEPTIDES INHIBITING PROTEIN PHOSPHATASE 1-MEDIATED DEPHOSPHORYLATION OF PHOSPHOLAMBAN AND A NUCLEOTIDES ENCODING CCN5 PROTEIN OR FRAGMENTS THEREOF AND USE THEREOF. Applicant: BethphaGen Inc. The sequence listing filed with the application follows.

SEQUENCE LISTING (41 sequences)

SEQ ID NO: 1 - DNA, 69 bp, synthetic construct
  source 1..69: mol_type = other DNA; note = Signal peptide 1
atgtggtggcgcctttggtggctccttttgttgctgttgttgttgtggcctatggtgtgggccaagctg

SEQ ID NO: 2 - DNA, 99 bp, synthetic construct
  source 1..99: mol_type = other DNA; note = TATm3
tatgcaagagccgctgcaagacaggccagagcatatgcgagggcagctgctagacaggctagagcttatgctagagcagctgccaggcaggctagagct

SEQ ID NO: 3 - DNA, 33 bp, synthetic construct
  source 1..33: mol_type = other DNA; note = TAT1
tatgcaagagccgctgcaagacaggccagagca

SEQ ID NO: 4 - DNA, 33 bp, synthetic construct
  source 1..33: mol_type = other DNA; note = TAT2
tatgcgagggcagctgctagacaggctagagct

SEQ ID NO: 5 - DNA, 33 bp, synthetic construct
  source 1..33: mol_type = other DNA; note = TAT3
tatgctagagcagctgccaggcaggctagagct

SEQ ID NO: 6 - skipped

SEQ ID NO: 7 - DNA, 27 bp, synthetic construct
  source 1..27: mol_type = other DNA; note = SE (Decoy peptide 1)
agagccgagaccatcgaaatgccacaa

SEQ ID NO: 8 - skipped

SEQ ID NO: 9 - DNA, 27 bp, synthetic construct
  source 1..27: mol_type = other DNA; note = SE (Decoy peptide 2)
cgggccgagacaatagaaatgcctcag

SEQ ID NO: 10 - skipped

SEQ ID NO: 11 - DNA, 66 bp, synthetic construct
  source 1..66: mol_type = other DNA; note = P2A sequence
ggaagcggcgctactaacttctccctccttaaacaagccggagacgtggaagagaatccaggtccc

SEQ ID NO: 12 - DNA, 69 bp, synthetic construct
  source 1..69: mol_type = other DNA; note = Signal peptide 2
atgcgtggtactcctaaaacccatctgctggctttttctctgctgtgtctgctgagcaaagttcgtact

SEQ ID NO: 13 - DNA, 684 bp, synthetic construct
  source 1..684: mol_type = other DNA; note = CCN5 w/o signal peptide
cagctgtgcccgaccccgtgtacttgtccatggccaccaccgcgttgtcctctgggtgtacctctggttctggacggttgcggctgttgtcgtgtttgcgcccgtcgtctgggcgaaccttgtgatcagctgcacgtttgcgacgcttcccagggtctggtttgccagcctggtgctggtcctggtggtcgtggtgcactgtgcctgctggctgaagacgactcttcttgtgaagtaaacggtcgtctgtaccgtgaaggtgagaccttccagccacattgctctattcgctgccgctgcgaagatggcggctttacttgtgttcctctgtgctccgaagacgttcgtctgccgtcttgggattgtcctcatccgcgtcgtgttgaagtgctgggcaaatgctgcccggaatgggtttgcggtcaaggtggtggtctgggtactcaaccgctgccggctcagggtccacaattctctggcctggttagcagcctgccgcctggtgttccttgtccagaatggagcacggcttggggcccttgttctaccacttgcggcctgggtatggctacccgtgtttccaaccagaaccgtttttgtcgtctggaaacccagcgtcgtctgtgtctgagccgtccgtgtccgccatctcgtggtcgttccccacagaactccgctttctga

SEQ ID NO: 14 - protein, 23 aa, synthetic construct
  source 1..23: note = Signal peptide 1
MWWRLWWLLLLLLLLWPMVWAKL

SEQ ID NO: 15 - protein, 33 aa, synthetic construct
  source 1..33: note = TATm3
YARAAARQARAYARAAARQARAYARAAARQARA

SEQ ID NO: 16 - protein, 11 aa, synthetic construct
  source 1..11: note = TAT
YARAAARQARA

SEQ ID NO: 17 - skipped

SEQ ID NO: 18 - protein, 9 aa, synthetic construct
  source 1..9: note = SE1 (Decoy peptide)
RAETIEMPQ

SEQ ID NO: 19 - protein, 9 aa, synthetic construct
  source 1..9: note = SE2 (Decoy peptide)
RASEIEMPQ

SEQ ID NO: 20 - protein, 9 aa, synthetic construct
  source 1..9: note = SE3 (Decoy peptide)
RADTIEMPQ

SEQ ID NO: 21 - protein, 8 aa, synthetic construct
  source 1..8: note = SE4 (Decoy peptide)
AETIEMPQ

SEQ ID NO: 22 - protein, 7 aa, synthetic construct
  source 1..7: note = SE5 (Decoy peptide)
RAETIEM

SEQ ID NO: 23 - protein, 6 aa, synthetic construct
  source 1..6: note = SE6 (Decoy peptide)
RAETIE

SEQ ID NO: 24 - protein, 22 aa, synthetic construct
  source 1..22: note = P2A sequence
GSGATNFSLLKQAGDVEENPGP

SEQ ID NO: 25 - protein, 23 aa, synthetic construct
  source 1..23: note = Signal peptide 2
MRGTPKTHLLAFSLLCLLSKVRT

SEQ ID NO: 26 - protein, 227 aa, synthetic construct
  source 1..227: note = CCN5 w/o signal peptide
QLCPTPCTCPWPPPRCPLGVPLVLDGCGCCRVCARRLGEPCDQLHVCDASQGLVCQPGAGPGGRGALCLLAEDDSSCEVNGRLYREGETFQPHCSIRCRCEDGGFTCVPLCSEDVRLPSWDCPHPRRVEVLGKCCPEWVCGQGGGLGTQPLPAQGPQFSGLVSSLPPGVPCPEWSTAWGPCSTTCGLGMATRVSNQNRFCRLETQRRLCLSRPCPPSRGRSPQNSAF

SEQ ID NO: 27 - protein, 52 aa, synthetic construct
  source 1..52: note = PLB_WT
MEKVQYLTRSAIRRASTIEMPQQARQKLQNLFINFCLILICLLLICIIVMLL

SEQ ID NO: 28 - protein, 9 aa, synthetic construct
  source 1..9: note = PLB WT_SE
RASTIEMPQ

SEQ ID NO: 29 - DNA, 22 bp, synthetic construct
  source 1..22: mol_type = other DNA; note = human alpha-SMA_F
gcccagccaagcactgtcagga

SEQ ID NO: 30 - DNA, 23 bp, synthetic construct
  source 1..23: mol_type = other DNA; note = human alpha-SMA_R
tcccaccatcaccccctgatgtc

SEQ ID NO: 31 - DNA, 22 bp, synthetic construct
  source 1..22: mol_type = other DNA; note = human Fibronectin_F
ctggccgaaaatacattgtaaa

SEQ ID NO: 32 - DNA, 18 bp, synthetic construct
  source 1..18: mol_type = other DNA; note = human Fibronectin_R
ccacagtcgggtcaggag

SEQ ID NO: 33 - DNA, 20 bp, synthetic construct
  source 1..20: mol_type = other DNA; note = human Vimentin_F
gagaactttgccgttgaagc

SEQ ID NO: 34 - DNA, 20 bp, synthetic construct
  source 1..20: mol_type = other DNA; note = human Vimentin_R
cgtgatgctgagaagtttcg

SEQ ID NO: 35 - DNA, 21 bp, synthetic construct
  source 1..21: mol_type = other DNA; note = 18s rRNA_F
taacgaacgagactctggcat

SEQ ID NO: 36 - DNA, 22 bp, synthetic construct
  source 1..22: mol_type = other DNA; note = 18s rRNA_R
cggacatctaagggcatcacag

SEQ ID NO: 37 - protein, 22 aa, synthetic construct
  source 1..22: note = Signal peptide 1 w/o start codon
WWRLWWLLLLLLLLWPMVWAKL

SEQ ID NO: 38 - protein, 11 aa, synthetic construct
  source 1..11: note = WT TAT
YGRKKRRQRRR

SEQ ID NO: 39 - protein, 21 aa, synthetic construct
  source 1..21: note = T2A
GSGEGRGSLLTCGDVEENPGP

SEQ ID NO: 40 - protein, 23 aa, synthetic construct
  source 1..23: note = E2A
GSGQCTNYALLKLAGDVESNPGP

SEQ ID NO: 41 - protein, 25 aa, synthetic construct
  source 1..25: note = F2A
GSGVKQTLNFDLLKLAGDVESNPGP